European Patent Application EP 4 653 529 A1, published November 26, 2025. Title: RNA HAVING LARIAT-CAP STRUCTURE FOR IMPROVING INTRACELLULAR STABILITY AND BIOGENESIS OF MRNA, AND USE THEREOF. Applicant: Korea Advanced Institute of Science and Technology. Application KR. The sequence listing filed with the application follows.

SEQUENCE LISTING (4 sequences)

SEQ ID NO: 1 - DNA, 188 bp, Didymium iridis
  source 1..188: mol_type = genomic DNA
ggttgggttgggaagtatcatggctaatcaccatgatgcaatcgggttgaacacttaattgggttaaaacggtgggggacgatcccgtaacatccgtcctaacggcgacagactgcacggccctgcctcttaggtgtgttcaatgaacagtcgttccgaaaggaagcatccggtatcccaagacaatc

SEQ ID NO: 2 - DNA, 200 bp, Allovahlkampfia spelaea
  source 1..200: mol_type = genomic DNA
gggcgactttctttttctcttgtgcaatggggtttatgagttaattagccaaaacgggaccttaaaaaggtgtaagtaaccgtactaagttcgtaagaacggaatgtctagagactacacggctgagcgatttagctctcataaatggatagtcctcagtataccatctgagcatcccatacaaaatggttaaatatttc

SEQ ID NO: 3 - DNA, 222 bp, Naegleria pringsheimi
  source 1..222: mol_type = genomic DNA
ggtccctgttattgaggacgttttagtgtgcaatggggttcacacctttatttgccaaaacgggacctctgttgaggttataaaattctaacgaattgaatattccgtactaaggatttaatccggaacgtctagagactacacggcaaaccatattggtggtgtgaatggatagtccctagtaaccatctaggcatcccatacaaaatggtaaccataaaa

SEQ ID NO: 4 - DNA, 744 bp, Artificial Sequence
  source 1..744: mol_type = genomic DNA
ttaaaacagcctgtgggttgatcccacccacaggcccattgggcgctagcactctggtatcacggtacctttgtgcgcctgttttataccccctcccccaactgtaacttagaagtaacacacaccgatcaacagtcagcgtggcacaccagccacgttttgatcaagcacttctgttaccccggactgagtatcaatagactgctcacgcggttgaaggagaaagcgttcgttatccggccaactacttcgaaaaacctagtaacaccgtggaagttgcagagtgtttcgctcagcactaccccagtgtagatcaggtcgatgagtcaccgcattccccacgggcgaccgtggcggtggctgcgttggcggcctgcccatggggaaacccatgggacgctctaatacagacatggtgcgaagagtctattgagctagttggtagtcctccggcccctgaatgcggctaatcctaactgcggagcacacaccctcaagccagagggcagtgtgtcgtaacgggcaactctgcagcggaaccgactactttgggtgtccgtgtttcattttattcctatactggctgcttatggtgacaattgagagatcgttaccatatagctattggattggccatccggtgactaatagagctattatatatccctttgttgggtttataccacttagcttgaaagaggttaaaacattacaattcattgttaagttgaatacagcaaaatg